European Patent Application EP 4 763 975 A1, published June 24, 2026. Title: Method for producing small intestine tissue. Applicant: Kyoto University. The sequence listing filed with the application follows.

SEQUENCE LISTING (62 sequences)

SEQ ID NO: 1 - DNA, 23 bp, synthetic construct
  source 1..23: mol_type = other DNA
  misc_feature 1..23: note = PCR Primer for GAPDH (Forward)
ggtggtctcctctgacttcaaca

SEQ ID NO: 2 - DNA, 19 bp, synthetic construct
  source 1..19: mol_type = other DNA
  misc_feature 1..19: note = PCR Primer for GAPDH (Reverse)
gtggtcgttgagggcaatg

SEQ ID NO: 3 - DNA, 23 bp, synthetic construct
  source 1..23: mol_type = other DNA
  misc_feature 1..23: note = PCR Primer for ALB (Forward)
tgcaactcttcgtgaaacctatg

SEQ ID NO: 4 - DNA, 21 bp, synthetic construct
  source 1..21: mol_type = other DNA
  misc_feature 1..21: note = PCR Primer for ALB (Reverse)
acatcaacctctggtctcacc

SEQ ID NO: 5 - DNA, 19 bp, synthetic construct
  source 1..19: mol_type = other DNA
  misc_feature 1..19: note = PCR Primer for VIL1 (Forward)
ctgagcgcccaagtcaaag

SEQ ID NO: 6 - DNA, 21 bp, synthetic construct
  source 1..21: mol_type = other DNA
  misc_feature 1..21: note = PCR Primer for VIL1 (Reverse)
agcagtcaccatcgaagaagc

SEQ ID NO: 7 - DNA, 21 bp, synthetic construct
  source 1..21: mol_type = other DNA
  misc_feature 1..21: note = PCR Primer for SI (Forward)
tccagctactactcgtgtgac

SEQ ID NO: 8 - DNA, 22 bp, synthetic construct
  source 1..22: mol_type = other DNA
  misc_feature 1..22: note = PCR Primer for SI (Reverse)
ccctctgttgggaattgttctg

SEQ ID NO: 9 - DNA, 22 bp, synthetic construct
  source 1..22: mol_type = other DNA
  misc_feature 1..22: note = PCR Primer for LYZ (Forward)
cttgtcctcctttctgttacgg

SEQ ID NO: 10 - DNA, 20 bp, synthetic construct
  source 1..20: mol_type = other DNA
  misc_feature 1..20: note = PCR Primer for LYZ (Reverse)
cccctgtagccatccattcc

SEQ ID NO: 11 - DNA, 19 bp, synthetic construct
  source 1..19: mol_type = other DNA
  misc_feature 1..19: note = PCR Primer for MUC2 (Forward)
gagggcagaacccgaaacc

SEQ ID NO: 12 - DNA, 21 bp, synthetic construct
  source 1..21: mol_type = other DNA
  misc_feature 1..21: note = PCR Primer for MUC2 (Reverse)
ggcgaagttgtagtcgcagag

SEQ ID NO: 13 - DNA, 22 bp, synthetic construct
  source 1..22: mol_type = other DNA
  misc_feature 1..22: note = PCR Primer for CHGA (Forward)
taaaggggataccgaggtgatg

SEQ ID NO: 14 - DNA, 22 bp, synthetic construct
  source 1..22: mol_type = other DNA
  misc_feature 1..22: note = PCR Primer for CHGA (Reverse)
tcggagtgtctcaaaacattcc

SEQ ID NO: 15 - DNA, 20 bp, synthetic construct
  source 1..20: mol_type = other DNA
  misc_feature 1..20: note = PCR Primer for LGR5 (Forward)
ctcccaggtctggtgtgttg

SEQ ID NO: 16 - DNA, 20 bp, synthetic construct
  source 1..20: mol_type = other DNA
  misc_feature 1..20: note = PCR Primer for LGR5 (Reverse)
gtgaagacgctgaggttgga

SEQ ID NO: 17 - DNA, 20 bp, synthetic construct
  source 1..20: mol_type = other DNA
  misc_feature 1..20: note = PCR Primer for OSTA (Forward)
ctgggctccattgccatctt

SEQ ID NO: 18 - DNA, 21 bp, synthetic construct
  source 1..21: mol_type = other DNA
  misc_feature 1..21: note = PCR Primer for OSTA (Reverse)
cacggcataaaacgaggtgat

SEQ ID NO: 19 - DNA, 21 bp, synthetic construct
  source 1..21: mol_type = other DNA
  misc_feature 1..21: note = PCR Primer for OSTB (Forward)
tccaggcaagcagaaaagaaa

SEQ ID NO: 20 - DNA, 21 bp, synthetic construct
  source 1..21: mol_type = other DNA
  misc_feature 1..21: note = PCR Primer for OSTB (Reverse)
actgacagcacatctctctct

SEQ ID NO: 21 - DNA, 20 bp, synthetic construct
  source 1..20: mol_type = other DNA
  misc_feature 1..20: note = PCR Primer for ASBT (Forward)
gggagagggacttcctcaag

SEQ ID NO: 22 - DNA, 20 bp, synthetic construct
  source 1..20: mol_type = other DNA
  misc_feature 1..20: note = PCR Primer for ASBT (Reverse)
ccctgaccatggtgcttact

SEQ ID NO: 23 - DNA, 21 bp, synthetic construct
  source 1..21: mol_type = other DNA
  misc_feature 1..21: note = PCR Primer for FGF19 (Forward)
cggaggaagactgtgctttcg

SEQ ID NO: 24 - DNA, 22 bp, synthetic construct
  source 1..22: mol_type = other DNA
  misc_feature 1..22: note = PCR Primer for FGF19 (Reverse)
ctcggatcggtacacattgtag

SEQ ID NO: 25 - DNA, 21 bp, synthetic construct
  source 1..21: mol_type = other DNA
  misc_feature 1..21: note = PCR Primer for CYP3A4 (Forward)
aagtcgcctcgaagatacaca

SEQ ID NO: 26 - DNA, 21 bp, synthetic construct
  source 1..21: mol_type = other DNA
  misc_feature 1..21: note = PCR Primer for CYP3A4 (Reverse)
aaggagagaacactgctcgtg

SEQ ID NO: 27 - DNA, 22 bp, synthetic construct
  source 1..22: mol_type = other DNA
  misc_feature 1..22: note = PCR Primer for CDX2 (Forward)
tccgtgtacaccactcgatatt

SEQ ID NO: 28 - DNA, 19 bp, synthetic construct
  source 1..19: mol_type = other DNA
  misc_feature 1..19: note = PCR Primer for CDX2 (Reverse)
ggaacctgtgcgagtggat

SEQ ID NO: 29 - DNA, 20 bp, synthetic construct
  source 1..20: mol_type = other DNA
  misc_feature 1..20: note = PCR Primer for REG4 (Forward)
ctgctcctattgctgagctg

SEQ ID NO: 30 - DNA, 23 bp, synthetic construct
  source 1..23: mol_type = other DNA
  misc_feature 1..23: note = PCR Primer for REG4 (Reverse)
ggacttgtggtaaaaccatccag

SEQ ID NO: 31 - DNA, 23 bp, synthetic construct
  source 1..23: mol_type = other DNA
  misc_feature 1..23: note = PCR Primer for GP2 (Forward)
aatcaaacccatgccatctacaa

SEQ ID NO: 32 - DNA, 21 bp, synthetic construct
  source 1..21: mol_type = other DNA
  misc_feature 1..21: note = PCR Primer for GP2 (Reverse)
cacactgacgttcagggaact

SEQ ID NO: 33 - DNA, 20 bp, synthetic construct
  source 1..20: mol_type = other DNA
  misc_feature 1..20: note = PCR Primer for DCLK1 (Forward)
acttcgacgagcgggataag

SEQ ID NO: 34 - DNA, 21 bp, synthetic construct
  source 1..21: mol_type = other DNA
  misc_feature 1..21: note = PCR Primer for DCLK1 (Reverse)
gggcctcaaaagatcggaacc

SEQ ID NO: 35 - DNA, 22 bp, synthetic construct
  source 1..22: mol_type = other DNA
  misc_feature 1..22: note = PCR Primer for HCoV-229E (Forward)
gtcgtcagggtagaatacctta

SEQ ID NO: 36 - DNA, 19 bp, synthetic construct
  source 1..19: mol_type = other DNA
  misc_feature 1..19: note = PCR Primer for HCoV-229E (Reverse)
cccgtttgcgctttctagt

SEQ ID NO: 37 - DNA, 22 bp, synthetic construct
  source 1..22: mol_type = other DNA
  misc_feature 1..22: note = PCR Primer for IL-8 (Forward)
ttttgccaaggagtgctaaaga

SEQ ID NO: 38 - DNA, 21 bp, synthetic construct
  source 1..21: mol_type = other DNA
  misc_feature 1..21: note = PCR Primer for IL-8 (Reverse)
aaccctctgcacccagttttc

SEQ ID NO: 39 - DNA, 23 bp, synthetic construct
  source 1..23: mol_type = other DNA
  misc_feature 1..23: note = PCR Primer for IL1B (Forward)
atgatggcttattacagtggcaa

SEQ ID NO: 40 - DNA, 20 bp, synthetic construct
  source 1..20: mol_type = other DNA
  misc_feature 1..20: note = PCR Primer for IL1B (Reverse)
gtcggagattcgtagctgga

SEQ ID NO: 41 - DNA, 21 bp, synthetic construct
  source 1..21: mol_type = other DNA
  misc_feature 1..21: note = PCR Primer for GAPDH (Forward)
ggagcgagatccctccaaaat

SEQ ID NO: 42 - DNA, 23 bp, synthetic construct
  source 1..23: mol_type = other DNA
  misc_feature 1..23: note = PCR Primer for GAPDH (Reverse)
ggctgttgtcatacttctcatgg

SEQ ID NO: 43 - DNA, 21 bp, synthetic construct
  source 1..21: mol_type = other DNA
  misc_feature 1..21: note = PCR Primer for CYP3A4 (Forward)
aagtcgcctcgaagatacaca

SEQ ID NO: 44 - DNA, 21 bp, synthetic construct
  source 1..21: mol_type = other DNA
  misc_feature 1..21: note = PCR Primer for CYP3A4 (Reverse)
aaggagagaacactgctcgtg

SEQ ID NO: 45 - DNA, 20 bp, synthetic construct
  source 1..20: mol_type = other DNA
  misc_feature 1..20: note = PCR Primer for UGT1A1 (Forward)
taagtggctaccccaaaacg

SEQ ID NO: 46 - DNA, 20 bp, synthetic construct
  source 1..20: mol_type = other DNA
  misc_feature 1..20: note = PCR Primer for UGT1A1 (Reverse)
gctttgcattgtccatctga

SEQ ID NO: 47 - DNA, 22 bp, synthetic construct
  source 1..22: mol_type = other DNA
  misc_feature 1..22: note = PCR Primer for SULT1B1 (Forward)
ttgaacagttccatagcagacc

SEQ ID NO: 48 - DNA, 23 bp, synthetic construct
  source 1..23: mol_type = other DNA
  misc_feature 1..23: note = PCR Primer for SULT1B1 (Reverse)
cagggagagtcatttccaacatt

SEQ ID NO: 49 - DNA, 20 bp, synthetic construct
  source 1..20: mol_type = other DNA
  misc_feature 1..20: note = PCR Primer for ABCB1/MDR1 (Forward)
gccaaagccaaaatatcagc

SEQ ID NO: 50 - DNA, 20 bp, synthetic construct
  source 1..20: mol_type = other DNA
  misc_feature 1..20: note = PCR Primer for ABCB1/MDR1 (Reverse)
ttccaatgtgttcggcatta

SEQ ID NO: 51 - DNA, 22 bp, synthetic construct
  source 1..22: mol_type = other DNA
  misc_feature 1..22: note = PCR Primer for ABCC1/MRP1 (Forward)
ctctatctctcccgacatgacc

SEQ ID NO: 52 - DNA, 21 bp, synthetic construct
  source 1..21: mol_type = other DNA
  misc_feature 1..21: note = PCR Primer for ABCC1/MRP1 (Reverse)
agcagacgatccacagcaaaa

SEQ ID NO: 53 - DNA, 22 bp, synthetic construct
  source 1..22: mol_type = other DNA
  misc_feature 1..22: note = PCR Primer for ABCC2/MRP2 (Forward)
tgagcaagtttgaaacgcacat

SEQ ID NO: 54 - DNA, 21 bp, synthetic construct
  source 1..21: mol_type = other DNA
  misc_feature 1..21: note = PCR Primer for ABCC2/MRP2 (Reverse)
agctcttctcctgccgtctct

SEQ ID NO: 55 - DNA, 21 bp, synthetic construct
  source 1..21: mol_type = other DNA
  misc_feature 1..21: note = PCR Primer for ABCG2/BCRP (Forward)
tgcaacatgtactggcgaaga

SEQ ID NO: 56 - DNA, 18 bp, synthetic construct
  source 1..18: mol_type = other DNA
  misc_feature 1..18: note = PCR Primer for ABCG2/BCRP (Reverse)
tcttccacaagccccagg

SEQ ID NO: 57 - DNA, 20 bp, synthetic construct
  source 1..20: mol_type = other DNA
  misc_feature 1..20: note = PCR Primer for SLCO2B1/OATP2B1 (Forward)
tttgcccacaacagcaactc

SEQ ID NO: 58 - DNA, 23 bp, synthetic construct
  source 1..23: mol_type = other DNA
  misc_feature 1..23: note = PCR Primer for SLCO2B1/OATP2B1 (Reverse)
tggttaatgtccacataaaggcg

SEQ ID NO: 59 - DNA, 21 bp, synthetic construct
  source 1..21: mol_type = other DNA
  misc_feature 1..21: note = PCR Primer for SLC15A1/PEPT1 (Forward)
tctttggttatcccctgagca

SEQ ID NO: 60 - DNA, 21 bp, synthetic construct
  source 1..21: mol_type = other DNA
  misc_feature 1..21: note = PCR Primer for SLC15A1/PEPT1 (Reverse)
ggcggtggacaggttatcatc

SEQ ID NO: 61 - DNA, 20 bp, synthetic construct
  source 1..20: mol_type = other DNA
  misc_feature 1..20: note = PCR Primer for FABP2 (Forward)
atggcgtttgacagcacttg

SEQ ID NO: 62 - DNA, 23 bp, synthetic construct
  source 1..23: mol_type = other DNA
  misc_feature 1..23: note = PCR Primer for FABP2 (Reverse)
tcagttccgtctgctagattgta